European Patent Application EP 4 792 837 A1, published August 19, 2026. Title: CONJUGATE, DRUG CONJUGATE AND COMPOSITION, AND PREPARATION METHOD AND USE. Applicant: SUZHOU RIBO LIFE SCIENCE CO., LTD. Application CN. The sequence listing filed with the application follows.

SEQUENCE LISTING (44 sequences)

SEQ ID NO: 1 - RNA, 21 nt, synthetic construct
  source 1..21: mol_type = other RNA
  misc_feature 1..21: note = synthetic sequence
ctgcttcagacgtgttagctt

SEQ ID NO: 2 - RNA, 22 nt, synthetic construct
  source 1..22: mol_type = other RNA
  misc_feature 1..22: note = synthetic sequence
ctgagttcagacgtgttgctct

SEQ ID NO: 3 - RNA, 32 nt, synthetic construct
  source 1..32: mol_type = other RNA
  misc_feature 1..32: note = synthetic sequence
tctatggctgccgatctggtctccatgtacgt

SEQ ID NO: 4 - RNA, 21 nt, synthetic construct
  source 1..21: mol_type = other RNA
  misc_feature 1: note = n is cu, uc or ac
  misc_feature 10: note = n is a, u, c, or g
  misc_feature 11: note = n is a, u, c or g
  misc_feature 12: note = n is a, u, c, or g
  misc_feature 13: note = n is a motif composed of u, c, or g, or two of them
  misc_feature 16: note = n is u, cu or uu
  misc_feature 21: note = n is u, uu, or uuN8,N8 is a motif composed of 1-15 nucleotides
  misc_feature 1..21: note = synthetic sequence
nggagttcannnntgngctcn

SEQ ID NO: 5 - RNA, 24 nt, synthetic construct
  source 1..24: mol_type = other RNA
  misc_feature 1..24: note = synthetic sequence
ctggagttcagacgtgttgctctt

SEQ ID NO: 6 - RNA, 24 nt, synthetic construct
  source 1..24: mol_type = other RNA
  misc_feature 1..24: note = synthetic sequence
ctggagttcagacgttgtgctctt

SEQ ID NO: 7 - RNA, 24 nt, synthetic construct
  source 1..24: mol_type = other RNA
  misc_feature 1..24: note = synthetic sequence
ctggagttcagaccgtgtgctctt

SEQ ID NO: 8 - RNA, 23 nt, synthetic construct
  source 1..23: mol_type = other RNA
  misc_feature 1..23: note = synthetic sequence
ctggagttcagacgtgttgctct

SEQ ID NO: 9 - RNA, 24 nt, synthetic construct
  source 1..24: mol_type = other RNA
  misc_feature 1..24: note = synthetic sequence
acggagttcagacgtgttgctctt

SEQ ID NO: 10 - RNA, 24 nt, synthetic construct
  source 1..24: mol_type = other RNA
  misc_feature 1..24: note = synthetic sequence
ctggagttcactactgttgctctt

SEQ ID NO: 11 - RNA, 24 nt, synthetic construct
  source 1..24: mol_type = other RNA
  misc_feature 1..24: note = synthetic sequence
ctggagttcagttgtgttgctctt

SEQ ID NO: 12 - RNA, 32 nt, synthetic construct
  source 1..32: mol_type = other RNA
  misc_feature 1..32: note = synthetic sequence
ctggagttcagacgtgttgctcttccgatctc

SEQ ID NO: 13 - RNA, 32 nt, synthetic construct
  source 1..32: mol_type = other RNA
  misc_feature 1..32: note = synthetic sequence
ctggagttcagacgttgtgctcttccgatctc

SEQ ID NO: 14 - RNA, 32 nt, synthetic construct
  source 1..32: mol_type = other RNA
  misc_feature 1..32: note = synthetic sequence
ctggagttcagaccgtgtgctcttccgatctc

SEQ ID NO: 15 - RNA, 32 nt, synthetic construct; identical to SEQ ID NO: 12
  source 1..32: mol_type = other RNA
  modified_base 1: mod_base = OTHER; note = Fluorinated modification
  modified_base 2: mod_base = OTHER; note = Fluorinated modification
  modified_base 7: mod_base = OTHER; note = Fluorinated modification
  modified_base 8: mod_base = OTHER; note = Fluorinated modification
  modified_base 9: mod_base = OTHER; note = Fluorinated modification
  modified_base 13: mod_base = OTHER; note = Fluorinated modification
  modified_base 15: mod_base = OTHER; note = Fluorinated modification
  modified_base 17: mod_base = OTHER; note = Fluorinated modification
  modified_base 18: mod_base = OTHER; note = Fluorinated modification
  modified_base 20: mod_base = OTHER; note = Fluorinated modification
  modified_base 21: mod_base = OTHER; note = Fluorinated modification
  modified_base 22: mod_base = OTHER; note = Fluorinated modification
  modified_base 23: mod_base = OTHER; note = Fluorinated modification
  modified_base 24: mod_base = OTHER; note = Fluorinated modification
  modified_base 25: mod_base = OTHER; note = Fluorinated modification
  modified_base 26: mod_base = OTHER; note = Fluorinated modification
  modified_base 29: mod_base = OTHER; note = Fluorinated modification
  modified_base 30: mod_base = OTHER; note = Fluorinated modification
  modified_base 31: mod_base = OTHER; note = Fluorinated modification
  modified_base 32: mod_base = OTHER; note = Fluorinated modification
  misc_feature 1..32: note = synthetic sequence

SEQ ID NO: 16 - RNA, 24 nt, synthetic construct
  source 1..24: mol_type = other RNA
  modified_base 1: mod_base = OTHER; note = Fluorinated modification
  modified_base 2: mod_base = OTHER; note = Fluorinated modification
  modified_base 7: mod_base = OTHER; note = Fluorinated modification
  modified_base 8: mod_base = OTHER; note = Fluorinated modification
  modified_base 9: mod_base = OTHER; note = Fluorinated modification
  modified_base 13: mod_base = OTHER; note = Fluorinated modification
  modified_base 15: mod_base = OTHER; note = Fluorinated modification
  modified_base 17: mod_base = OTHER; note = Fluorinated modification
  modified_base 18: mod_base = OTHER; note = Fluorinated modification
  modified_base 20: mod_base = OTHER; note = Fluorinated modification
  modified_base 21: mod_base = OTHER; note = Fluorinated modification
  modified_base 22: mod_base = OTHER; note = Fluorinated modification
  modified_base 23: mod_base = OTHER; note = Fluorinated modification
  modified_base 24: mod_base = OTHER; note = Fluorinated modification
  misc_feature 1..24: note = synthetic sequence
ctggagttcagacgtgttgctctt

SEQ ID NO: 17 - RNA, 32 nt, synthetic construct; identical to SEQ ID NO: 13
  source 1..32: mol_type = other RNA
  modified_base 1: mod_base = OTHER; note = Fluorinated modification
  modified_base 2: mod_base = OTHER; note = Fluorinated modification
  modified_base 7: mod_base = OTHER; note = Fluorinated modification
  modified_base 8: mod_base = OTHER; note = Fluorinated modification
  modified_base 9: mod_base = OTHER; note = Fluorinated modification
  modified_base 13: mod_base = OTHER; note = Fluorinated modification
  modified_base 15: mod_base = OTHER; note = Fluorinated modification
  modified_base 16: mod_base = OTHER; note = Fluorinated modification
  modified_base 18: mod_base = OTHER; note = Fluorinated modification
  modified_base 20: mod_base = OTHER; note = Fluorinated modification
  modified_base 21: mod_base = OTHER; note = Fluorinated modification
  modified_base 22: mod_base = OTHER; note = Fluorinated modification
  modified_base 23: mod_base = OTHER; note = Fluorinated modification
  modified_base 24: mod_base = OTHER; note = Fluorinated modification
  modified_base 25: mod_base = OTHER; note = Fluorinated modification
  modified_base 26: mod_base = OTHER; note = Fluorinated modification
  modified_base 29: mod_base = OTHER; note = Fluorinated modification
  modified_base 30: mod_base = OTHER; note = Fluorinated modification
  modified_base 31: mod_base = OTHER; note = Fluorinated modification
  modified_base 32: mod_base = OTHER; note = Fluorinated modification
  misc_feature 1..32: note = synthetic sequence

SEQ ID NO: 18 - RNA, 24 nt, synthetic construct
  source 1..24: mol_type = other RNA
  modified_base 1: mod_base = OTHER; note = Fluorinated modification
  modified_base 2: mod_base = OTHER; note = Fluorinated modification
  modified_base 7: mod_base = OTHER; note = Fluorinated modification
  modified_base 8: mod_base = OTHER; note = Fluorinated modification
  modified_base 9: mod_base = OTHER; note = Fluorinated modification
  modified_base 13: mod_base = OTHER; note = Fluorinated modification
  modified_base 15: mod_base = OTHER; note = Fluorinated modification
  modified_base 16: mod_base = OTHER; note = Fluorinated modification
  modified_base 18: mod_base = OTHER; note = Fluorinated modification
  modified_base 20: mod_base = OTHER; note = Fluorinated modification
  modified_base 21: mod_base = OTHER; note = Fluorinated modification
  modified_base 22: mod_base = OTHER; note = Fluorinated modification
  modified_base 23: mod_base = OTHER; note = Fluorinated modification
  modified_base 24: mod_base = OTHER; note = Fluorinated modification
  misc_feature 1..24: note = synthetic sequence
ctggagttcagacgttgtgctctt

SEQ ID NO: 19 - RNA, 32 nt, synthetic construct; identical to SEQ ID NO: 14
  source 1..32: mol_type = other RNA
  modified_base 1: mod_base = OTHER; note = Fluorinated modification
  modified_base 2: mod_base = OTHER; note = Fluorinated modification
  modified_base 7: mod_base = OTHER; note = Fluorinated modification
  modified_base 8: mod_base = OTHER; note = Fluorinated modification
  modified_base 9: mod_base = OTHER; note = Fluorinated modification
  modified_base 13: mod_base = OTHER; note = Fluorinated modification
  modified_base 14: mod_base = OTHER; note = Fluorinated modification
  modified_base 16: mod_base = OTHER; note = Fluorinated modification
  modified_base 18: mod_base = OTHER; note = Fluorinated modification
  modified_base 20: mod_base = OTHER; note = Fluorinated modification
  modified_base 21: mod_base = OTHER; note = Fluorinated modification
  modified_base 22: mod_base = OTHER; note = Fluorinated modification
  modified_base 23: mod_base = OTHER; note = Fluorinated modification
  modified_base 24: mod_base = OTHER; note = Fluorinated modification
  modified_base 25: mod_base = OTHER; note = Fluorinated modification
  modified_base 26: mod_base = OTHER; note = Fluorinated modification
  modified_base 29: mod_base = OTHER; note = Fluorinated modification
  modified_base 30: mod_base = OTHER; note = Fluorinated modification
  modified_base 31: mod_base = OTHER; note = Fluorinated modification
  modified_base 32: mod_base = OTHER; note = Fluorinated modification
  misc_feature 1..32: note = synthetic sequence

SEQ ID NO: 20 - RNA, 24 nt, synthetic construct
  source 1..24: mol_type = other RNA
  modified_base 1: mod_base = OTHER; note = Fluorinated modification
  modified_base 2: mod_base = OTHER; note = Fluorinated modification
  modified_base 7: mod_base = OTHER; note = Fluorinated modification
  modified_base 8: mod_base = OTHER; note = Fluorinated modification
  modified_base 9: mod_base = OTHER; note = Fluorinated modification
  modified_base 13: mod_base = OTHER; note = Fluorinated modification
  modified_base 14: mod_base = OTHER; note = Fluorinated modification
  modified_base 16: mod_base = OTHER; note = Fluorinated modification
  modified_base 18: mod_base = OTHER; note = Fluorinated modification
  modified_base 20: mod_base = OTHER; note = Fluorinated modification
  modified_base 21: mod_base = OTHER; note = Fluorinated modification
  modified_base 22: mod_base = OTHER; note = Fluorinated modification
  modified_base 23: mod_base = OTHER; note = Fluorinated modification
  modified_base 24: mod_base = OTHER; note = Fluorinated modification
  misc_feature 1..24: note = synthetic sequence
ctggagttcagaccgtgtgctctt

SEQ ID NO: 21 - RNA, 32 nt, synthetic construct; identical to SEQ ID NO: 12
  source 1..32: mol_type = other RNA
  modified_base 1: mod_base = OTHER; note = Methoxy modification
  modified_base 2: mod_base = OTHER; note = Methoxy modification
  modified_base 3: mod_base = OTHER; note = Methoxy modification
  modified_base 4: mod_base = OTHER; note = Methoxy modification
  modified_base 5: mod_base = OTHER; note = Methoxy modification
  modified_base 6: mod_base = OTHER; note = Methoxy modification
  modified_base 7: mod_base = OTHER; note = Methoxy modification
  modified_base 8: mod_base = OTHER; note = Methoxy modification
  modified_base 9: mod_base = OTHER; note = Methoxy modification
  modified_base 10: mod_base = OTHER; note = Methoxy modification
  modified_base 11: mod_base = OTHER; note = Methoxy modification
  modified_base 12: mod_base = OTHER; note = Methoxy modification
  modified_base 13: mod_base = OTHER; note = Methoxy modification
  modified_base 14: mod_base = OTHER; note = Methoxy modification
  modified_base 15: mod_base = OTHER; note = Methoxy modification
  modified_base 16: mod_base = OTHER; note = Methoxy modification
  modified_base 17: mod_base = OTHER; note = Methoxy modification
  modified_base 18: mod_base = OTHER; note = Methoxy modification
  modified_base 19: mod_base = OTHER; note = Methoxy modification
  modified_base 20: mod_base = OTHER; note = Methoxy modification
  modified_base 21: mod_base = OTHER; note = Methoxy modification
  modified_base 22: mod_base = OTHER; note = Methoxy modification
  modified_base 23: mod_base = OTHER; note = Methoxy modification
  modified_base 24: mod_base = OTHER; note = Methoxy modification
  modified_base 25: mod_base = OTHER; note = Methoxy modification
  modified_base 26: mod_base = OTHER; note = Methoxy modification
  modified_base 27: mod_base = OTHER; note = Methoxy modification
  modified_base 28: mod_base = OTHER; note = Methoxy modification
  modified_base 29: mod_base = OTHER; note = Methoxy modification
  modified_base 30: mod_base = OTHER; note = Methoxy modification
  modified_base 31: mod_base = OTHER; note = Methoxy modification
  modified_base 32: mod_base = OTHER; note = Methoxy modification
  misc_feature 1..32: note = synthetic sequence

SEQ ID NO: 22 - RNA, 24 nt, synthetic construct
  source 1..24: mol_type = other RNA
  modified_base 1: mod_base = OTHER; note = Methoxy modification
  modified_base 2: mod_base = OTHER; note = Methoxy modification
  modified_base 3: mod_base = OTHER; note = Methoxy modification
  modified_base 4: mod_base = OTHER; note = Methoxy modification
  modified_base 5: mod_base = OTHER; note = Methoxy modification
  modified_base 6: mod_base = OTHER; note = Methoxy modification
  modified_base 7: mod_base = OTHER; note = Methoxy modification
  modified_base 8: mod_base = OTHER; note = Methoxy modification
  modified_base 9: mod_base = OTHER; note = Methoxy modification
  modified_base 10: mod_base = OTHER; note = Methoxy modification
  modified_base 11: mod_base = OTHER; note = Methoxy modification
  modified_base 12: mod_base = OTHER; note = Methoxy modification
  modified_base 13: mod_base = OTHER; note = Methoxy modification
  modified_base 14: mod_base = OTHER; note = Methoxy modification
  modified_base 15: mod_base = OTHER; note = Methoxy modification
  modified_base 16: mod_base = OTHER; note = Methoxy modification
  modified_base 17: mod_base = OTHER; note = Methoxy modification
  modified_base 18: mod_base = OTHER; note = Methoxy modification
  modified_base 19: mod_base = OTHER; note = Methoxy modification
  modified_base 20: mod_base = OTHER; note = Methoxy modification
  modified_base 21: mod_base = OTHER; note = Methoxy modification
  modified_base 22: mod_base = OTHER; note = Methoxy modification
  modified_base 23: mod_base = OTHER; note = Methoxy modification
  modified_base 24: mod_base = OTHER; note = Methoxy modification
  misc_feature 1..24: note = synthetic sequence
ctggagttcagacgtgttgctctt

SEQ ID NO: 23 - RNA, 32 nt, synthetic construct; identical to SEQ ID NO: 13
  source 1..32: mol_type = other RNA
  modified_base 1: mod_base = OTHER; note = Methoxy modification
  modified_base 2: mod_base = OTHER; note = Methoxy modification
  modified_base 3: mod_base = OTHER; note = Methoxy modification
  modified_base 4: mod_base = OTHER; note = Methoxy modification
  modified_base 5: mod_base = OTHER; note = Methoxy modification
  modified_base 6: mod_base = OTHER; note = Methoxy modification
  modified_base 7: mod_base = OTHER; note = Methoxy modification
  modified_base 8: mod_base = OTHER; note = Methoxy modification
  modified_base 9: mod_base = OTHER; note = Methoxy modification
  modified_base 10: mod_base = OTHER; note = Methoxy modification
  modified_base 11: mod_base = OTHER; note = Methoxy modification
  modified_base 12: mod_base = OTHER; note = Methoxy modification
  modified_base 13: mod_base = OTHER; note = Methoxy modification
  modified_base 14: mod_base = OTHER; note = Methoxy modification
  modified_base 15: mod_base = OTHER; note = Methoxy modification
  modified_base 16: mod_base = OTHER; note = Methoxy modification
  modified_base 17: mod_base = OTHER; note = Methoxy modification
  modified_base 18: mod_base = OTHER; note = Methoxy modification
  modified_base 19: mod_base = OTHER; note = Methoxy modification
  modified_base 20: mod_base = OTHER; note = Methoxy modification
  modified_base 21: mod_base = OTHER; note = Methoxy modification
  modified_base 22: mod_base = OTHER; note = Methoxy modification
  modified_base 23: mod_base = OTHER; note = Methoxy modification
  modified_base 24: mod_base = OTHER; note = Methoxy modification
  modified_base 25: mod_base = OTHER; note = Methoxy modification
  modified_base 26: mod_base = OTHER; note = Methoxy modification
  modified_base 27: mod_base = OTHER; note = Methoxy modification
  modified_base 28: mod_base = OTHER; note = Methoxy modification
  modified_base 29: mod_base = OTHER; note = Methoxy modification
  modified_base 30: mod_base = OTHER; note = Methoxy modification
  modified_base 31: mod_base = OTHER; note = Methoxy modification
  modified_base 32: mod_base = OTHER; note = Methoxy modification
  misc_feature 1..32: note = synthetic sequence

SEQ ID NO: 24 - RNA, 24 nt, synthetic construct
  source 1..24: mol_type = other RNA
  modified_base 1: mod_base = OTHER; note = Methoxy modification
  modified_base 2: mod_base = OTHER; note = Methoxy modification
  modified_base 3: mod_base = OTHER; note = Methoxy modification
  modified_base 4: mod_base = OTHER; note = Methoxy modification
  modified_base 5: mod_base = OTHER; note = Methoxy modification
  modified_base 6: mod_base = OTHER; note = Methoxy modification
  modified_base 7: mod_base = OTHER; note = Methoxy modification
  modified_base 8: mod_base = OTHER; note = Methoxy modification
  modified_base 9: mod_base = OTHER; note = Methoxy modification
  modified_base 10: mod_base = OTHER; note = Methoxy modification
  modified_base 11: mod_base = OTHER; note = Methoxy modification
  modified_base 12: mod_base = OTHER; note = Methoxy modification
  modified_base 13: mod_base = OTHER; note = Methoxy modification
  modified_base 14: mod_base = OTHER; note = Methoxy modification
  modified_base 15: mod_base = OTHER; note = Methoxy modification
  modified_base 16: mod_base = OTHER; note = Methoxy modification
  modified_base 17: mod_base = OTHER; note = Methoxy modification
  modified_base 18: mod_base = OTHER; note = Methoxy modification
  modified_base 19: mod_base = OTHER; note = Methoxy modification
  modified_base 20: mod_base = OTHER; note = Methoxy modification
  modified_base 21: mod_base = OTHER; note = Methoxy modification
  modified_base 22: mod_base = OTHER; note = Methoxy modification
  modified_base 23: mod_base = OTHER; note = Methoxy modification
  modified_base 24: mod_base = OTHER; note = Methoxy modification
  misc_feature 1..24: note = synthetic sequence
ctggagttcagacgttgtgctctt

SEQ ID NO: 25 - RNA, 32 nt, synthetic construct; identical to SEQ ID NO: 14
  source 1..32: mol_type = other RNA
  modified_base 1: mod_base = OTHER; note = Methoxy modification
  modified_base 2: mod_base = OTHER; note = Methoxy modification
  modified_base 3: mod_base = OTHER; note = Methoxy modification
  modified_base 4: mod_base = OTHER; note = Methoxy modification
  modified_base 5: mod_base = OTHER; note = Methoxy modification
  modified_base 6: mod_base = OTHER; note = Methoxy modification
  modified_base 7: mod_base = OTHER; note = Methoxy modification
  modified_base 8: mod_base = OTHER; note = Methoxy modification
  modified_base 9: mod_base = OTHER; note = Methoxy modification
  modified_base 10: mod_base = OTHER; note = Methoxy modification
  modified_base 11: mod_base = OTHER; note = Methoxy modification
  modified_base 12: mod_base = OTHER; note = Methoxy modification
  modified_base 13: mod_base = OTHER; note = Methoxy modification
  modified_base 14: mod_base = OTHER; note = Methoxy modification
  modified_base 15: mod_base = OTHER; note = Methoxy modification
  modified_base 16: mod_base = OTHER; note = Methoxy modification
  modified_base 17: mod_base = OTHER; note = Methoxy modification
  modified_base 18: mod_base = OTHER; note = Methoxy modification
  modified_base 19: mod_base = OTHER; note = Methoxy modification
  modified_base 20: mod_base = OTHER; note = Methoxy modification
  modified_base 21: mod_base = OTHER; note = Methoxy modification
  modified_base 22: mod_base = OTHER; note = Methoxy modification
  modified_base 23: mod_base = OTHER; note = Methoxy modification
  modified_base 24: mod_base = OTHER; note = Methoxy modification
  modified_base 25: mod_base = OTHER; note = Methoxy modification
  modified_base 26: mod_base = OTHER; note = Methoxy modification
  modified_base 27: mod_base = OTHER; note = Methoxy modification
  modified_base 28: mod_base = OTHER; note = Methoxy modification
  modified_base 29: mod_base = OTHER; note = Methoxy modification
  modified_base 30: mod_base = OTHER; note = Methoxy modification
  modified_base 31: mod_base = OTHER; note = Methoxy modification
  modified_base 32: mod_base = OTHER; note = Methoxy modification
  misc_feature 1..32: note = synthetic sequence

SEQ ID NO: 26 - RNA, 24 nt, synthetic construct
  source 1..24: mol_type = other RNA
  modified_base 1: mod_base = OTHER; note = Methoxy modification
  modified_base 2: mod_base = OTHER; note = Methoxy modification
  modified_base 3: mod_base = OTHER; note = Methoxy modification
  modified_base 4: mod_base = OTHER; note = Methoxy modification
  modified_base 5: mod_base = OTHER; note = Methoxy modification
  modified_base 6: mod_base = OTHER; note = Methoxy modification
  modified_base 7: mod_base = OTHER; note = Methoxy modification
  modified_base 8: mod_base = OTHER; note = Methoxy modification
  modified_base 9: mod_base = OTHER; note = Methoxy modification
  modified_base 10: mod_base = OTHER; note = Methoxy modification
  modified_base 11: mod_base = OTHER; note = Methoxy modification
  modified_base 12: mod_base = OTHER; note = Methoxy modification
  modified_base 13: mod_base = OTHER; note = Methoxy modification
  modified_base 14: mod_base = OTHER; note = Methoxy modification
  modified_base 15: mod_base = OTHER; note = Methoxy modification
  modified_base 16: mod_base = OTHER; note = Methoxy modification
  modified_base 17: mod_base = OTHER; note = Methoxy modification
  modified_base 18: mod_base = OTHER; note = Methoxy modification
  modified_base 19: mod_base = OTHER; note = Methoxy modification
  modified_base 20: mod_base = OTHER; note = Methoxy modification
  modified_base 21: mod_base = OTHER; note = Methoxy modification
  modified_base 22: mod_base = OTHER; note = Methoxy modification
  modified_base 23: mod_base = OTHER; note = Methoxy modification
  modified_base 24: mod_base = OTHER; note = Methoxy modification
  misc_feature 1..24: note = synthetic sequence
ctggagttcagaccgtgtgctctt

SEQ ID NO: 27 - RNA, 23 nt, synthetic construct
  source 1..23: mol_type = other RNA
  modified_base 1: mod_base = OTHER; note = Methoxy modification
  modified_base 2: mod_base = OTHER; note = Methoxy modification
  modified_base 3: mod_base = OTHER; note = Methoxy modification
  modified_base 4: mod_base = OTHER; note = Methoxy modification
  modified_base 5: mod_base = OTHER; note = Methoxy modification
  modified_base 6: mod_base = OTHER; note = Methoxy modification
  modified_base 7: mod_base = OTHER; note = Methoxy modification
  modified_base 8: mod_base = OTHER; note = Methoxy modification
  modified_base 9: mod_base = OTHER; note = Methoxy modification
  modified_base 10: mod_base = OTHER; note = Methoxy modification
  modified_base 11: mod_base = OTHER; note = Methoxy modification
  modified_base 12: mod_base = OTHER; note = Methoxy modification
  modified_base 13: mod_base = OTHER; note = Methoxy modification
  modified_base 14: mod_base = OTHER; note = Methoxy modification
  modified_base 15: mod_base = OTHER; note = Methoxy modification
  modified_base 16: mod_base = OTHER; note = Methoxy modification
  modified_base 17: mod_base = OTHER; note = Methoxy modification
  modified_base 18: mod_base = OTHER; note = Methoxy modification
  modified_base 19: mod_base = OTHER; note = Methoxy modification
  modified_base 20: mod_base = OTHER; note = Methoxy modification
  modified_base 21: mod_base = OTHER; note = Methoxy modification
  modified_base 22: mod_base = OTHER; note = Methoxy modification
  modified_base 23: mod_base = OTHER; note = Methoxy modification
  misc_feature 1..23: note = synthetic sequence
ctggagttcagacgtgttgctct

SEQ ID NO: 28 - RNA, 22 nt, synthetic construct
  source 1..22: mol_type = other RNA
  modified_base 1: mod_base = OTHER; note = Methoxy modification
  modified_base 2: mod_base = OTHER; note = Methoxy modification
  modified_base 3: mod_base = OTHER; note = Methoxy modification
  modified_base 4: mod_base = OTHER; note = Methoxy modification
  modified_base 5: mod_base = OTHER; note = Methoxy modification
  modified_base 6: mod_base = OTHER; note = Methoxy modification
  modified_base 7: mod_base = OTHER; note = Methoxy modification
  modified_base 8: mod_base = OTHER; note = Methoxy modification
  modified_base 9: mod_base = OTHER; note = Methoxy modification
  modified_base 10: mod_base = OTHER; note = Methoxy modification
  modified_base 11: mod_base = OTHER; note = Methoxy modification
  modified_base 12: mod_base = OTHER; note = Methoxy modification
  modified_base 13: mod_base = OTHER; note = Methoxy modification
  modified_base 14: mod_base = OTHER; note = Methoxy modification
  modified_base 15: mod_base = OTHER; note = Methoxy modification
  modified_base 16: mod_base = OTHER; note = Methoxy modification
  modified_base 17: mod_base = OTHER; note = Methoxy modification
  modified_base 18: mod_base = OTHER; note = Methoxy modification
  modified_base 19: mod_base = OTHER; note = Methoxy modification
  modified_base 20: mod_base = OTHER; note = Methoxy modification
  modified_base 21: mod_base = OTHER; note = Methoxy modification
  modified_base 22: mod_base = OTHER; note = Methoxy modification
  misc_feature 1..22: note = synthetic sequence
ctgagttcagacgtgttgctct

SEQ ID NO: 29 - RNA, 21 nt, synthetic construct
  source 1..21: mol_type = other RNA
  modified_base 1: mod_base = OTHER; note = Methoxy modification
  modified_base 2: mod_base = OTHER; note = Methoxy modification
  modified_base 3: mod_base = OTHER; note = Methoxy modification
  modified_base 4: mod_base = OTHER; note = Methoxy modification
  modified_base 5: mod_base = OTHER; note = Methoxy modification
  modified_base 6: mod_base = OTHER; note = Methoxy modification
  modified_base 7: mod_base = OTHER; note = Methoxy modification
  modified_base 8: mod_base = OTHER; note = Methoxy modification
  modified_base 9: mod_base = OTHER; note = Methoxy modification
  modified_base 10: mod_base = OTHER; note = Methoxy modification
  modified_base 11: mod_base = OTHER; note = Methoxy modification
  modified_base 12: mod_base = OTHER; note = Methoxy modification
  modified_base 13: mod_base = OTHER; note = Methoxy modification
  modified_base 14: mod_base = OTHER; note = Methoxy modification
  modified_base 15: mod_base = OTHER; note = Methoxy modification
  modified_base 16: mod_base = OTHER; note = Methoxy modification
  modified_base 17: mod_base = OTHER; note = Methoxy modification
  modified_base 18: mod_base = OTHER; note = Methoxy modification
  modified_base 19: mod_base = OTHER; note = Methoxy modification
  modified_base 20: mod_base = OTHER; note = Methoxy modification
  modified_base 21: mod_base = OTHER; note = Methoxy modification
  misc_feature 1..21: note = synthetic sequence
ctgcttcagacgtgttagctt

SEQ ID NO: 30 - RNA, 24 nt, synthetic construct
  source 1..24: mol_type = other RNA
  modified_base 1: mod_base = OTHER; note = Methoxy modification
  modified_base 2: mod_base = OTHER; note = Methoxy modification
  modified_base 3: mod_base = OTHER; note = Methoxy modification
  modified_base 4: mod_base = OTHER; note = Methoxy modification
  modified_base 5: mod_base = OTHER; note = Methoxy modification
  modified_base 6: mod_base = OTHER; note = Methoxy modification
  modified_base 7: mod_base = OTHER; note = Methoxy modification
  modified_base 8: mod_base = OTHER; note = Methoxy modification
  modified_base 9: mod_base = OTHER; note = Methoxy modification
  modified_base 10: mod_base = OTHER; note = Methoxy modification
  modified_base 11: mod_base = OTHER; note = Methoxy modification
  modified_base 12: mod_base = OTHER; note = Methoxy modification
  modified_base 13: mod_base = OTHER; note = Methoxy modification
  modified_base 14: mod_base = OTHER; note = Methoxy modification
  modified_base 15: mod_base = OTHER; note = Methoxy modification
  modified_base 16: mod_base = OTHER; note = Methoxy modification
  modified_base 17: mod_base = OTHER; note = Methoxy modification
  modified_base 18: mod_base = OTHER; note = Methoxy modification
  modified_base 19: mod_base = OTHER; note = Methoxy modification
  modified_base 20: mod_base = OTHER; note = Methoxy modification
  modified_base 21: mod_base = OTHER; note = Methoxy modification
  modified_base 22: mod_base = OTHER; note = Methoxy modification
  modified_base 23: mod_base = OTHER; note = Methoxy modification
  modified_base 24: mod_base = OTHER; note = Methoxy modification
  misc_feature 1..24: note = synthetic sequence
acggagttcagacgtgttgctctt

SEQ ID NO: 31 - RNA, 24 nt, synthetic construct
  source 1..24: mol_type = other RNA
  modified_base 1: mod_base = OTHER; note = Methoxy modification
  modified_base 2: mod_base = OTHER; note = Methoxy modification
  modified_base 3: mod_base = OTHER; note = Methoxy modification
  modified_base 4: mod_base = OTHER; note = Methoxy modification
  modified_base 5: mod_base = OTHER; note = Methoxy modification
  modified_base 6: mod_base = OTHER; note = Methoxy modification
  modified_base 7: mod_base = OTHER; note = Methoxy modification
  modified_base 8: mod_base = OTHER; note = Methoxy modification
  modified_base 9: mod_base = OTHER; note = Methoxy modification
  modified_base 10: mod_base = OTHER; note = Methoxy modification
  modified_base 11: mod_base = OTHER; note = Methoxy modification
  modified_base 12: mod_base = OTHER; note = Methoxy modification
  modified_base 13: mod_base = OTHER; note = Methoxy modification
  modified_base 14: mod_base = OTHER; note = Methoxy modification
  modified_base 15: mod_base = OTHER; note = Methoxy modification
  modified_base 16: mod_base = OTHER; note = Methoxy modification
  modified_base 17: mod_base = OTHER; note = Methoxy modification
  modified_base 18: mod_base = OTHER; note = Methoxy modification
  modified_base 19: mod_base = OTHER; note = Methoxy modification
  modified_base 20: mod_base = OTHER; note = Methoxy modification
  modified_base 21: mod_base = OTHER; note = Methoxy modification
  modified_base 22: mod_base = OTHER; note = Methoxy modification
  modified_base 23: mod_base = OTHER; note = Methoxy modification
  modified_base 24: mod_base = OTHER; note = Methoxy modification
  misc_feature 1..24: note = synthetic sequence
ctggagttcactactgttgctctt

SEQ ID NO: 32 - RNA, 24 nt, synthetic construct
  source 1..24: mol_type = other RNA
  modified_base 1: mod_base = OTHER; note = Methoxy modification
  modified_base 2: mod_base = OTHER; note = Methoxy modification
  modified_base 3: mod_base = OTHER; note = Methoxy modification
  modified_base 4: mod_base = OTHER; note = Methoxy modification
  modified_base 5: mod_base = OTHER; note = Methoxy modification
  modified_base 6: mod_base = OTHER; note = Methoxy modification
  modified_base 7: mod_base = OTHER; note = Methoxy modification
  modified_base 8: mod_base = OTHER; note = Methoxy modification
  modified_base 9: mod_base = OTHER; note = Methoxy modification
  modified_base 10: mod_base = OTHER; note = Methoxy modification
  modified_base 11: mod_base = OTHER; note = Methoxy modification
  modified_base 12: mod_base = OTHER; note = Methoxy modification
  modified_base 13: mod_base = OTHER; note = Methoxy modification
  modified_base 14: mod_base = OTHER; note = Methoxy modification
  modified_base 15: mod_base = OTHER; note = Methoxy modification
  modified_base 16: mod_base = OTHER; note = Methoxy modification
  modified_base 17: mod_base = OTHER; note = Methoxy modification
  modified_base 18: mod_base = OTHER; note = Methoxy modification
  modified_base 19: mod_base = OTHER; note = Methoxy modification
  modified_base 20: mod_base = OTHER; note = Methoxy modification
  modified_base 21: mod_base = OTHER; note = Methoxy modification
  modified_base 22: mod_base = OTHER; note = Methoxy modification
  modified_base 23: mod_base = OTHER; note = Methoxy modification
  modified_base 24: mod_base = OTHER; note = Methoxy modification
  misc_feature 1..24: note = synthetic sequence
ctggagttcagttgtgttgctctt

SEQ ID NO: 33 - RNA, 32 nt, synthetic construct; identical to SEQ ID NO: 3
  source 1..32: mol_type = other RNA
  modified_base 1: mod_base = OTHER; note = Methoxy modification
  modified_base 2: mod_base = OTHER; note = Methoxy modification
  modified_base 3: mod_base = OTHER; note = Methoxy modification
  modified_base 4: mod_base = OTHER; note = Methoxy modification
  modified_base 5: mod_base = OTHER; note = Methoxy modification
  modified_base 6: mod_base = OTHER; note = Methoxy modification
  modified_base 7: mod_base = OTHER; note = Methoxy modification
  modified_base 8: mod_base = OTHER; note = Methoxy modification
  modified_base 9: mod_base = OTHER; note = Methoxy modification
  modified_base 10: mod_base = OTHER; note = Methoxy modification
  modified_base 11: mod_base = OTHER; note = Methoxy modification
  modified_base 12: mod_base = OTHER; note = Methoxy modification
  modified_base 13: mod_base = OTHER; note = Methoxy modification
  modified_base 14: mod_base = OTHER; note = Methoxy modification
  modified_base 15: mod_base = OTHER; note = Methoxy modification
  modified_base 16: mod_base = OTHER; note = Methoxy modification
  modified_base 17: mod_base = OTHER; note = Methoxy modification
  modified_base 18: mod_base = OTHER; note = Methoxy modification
  modified_base 19: mod_base = OTHER; note = Methoxy modification
  modified_base 20: mod_base = OTHER; note = Methoxy modification
  modified_base 21: mod_base = OTHER; note = Methoxy modification
  modified_base 22: mod_base = OTHER; note = Methoxy modification
  modified_base 23: mod_base = OTHER; note = Methoxy modification
  modified_base 24: mod_base = OTHER; note = Methoxy modification
  modified_base 25: mod_base = OTHER; note = Methoxy modification
  modified_base 26: mod_base = OTHER; note = Methoxy modification
  modified_base 27: mod_base = OTHER; note = Methoxy modification
  modified_base 28: mod_base = OTHER; note = Methoxy modification
  modified_base 29: mod_base = OTHER; note = Methoxy modification
  modified_base 30: mod_base = OTHER; note = Methoxy modification
  modified_base 31: mod_base = OTHER; note = Methoxy modification
  modified_base 32: mod_base = OTHER; note = Methoxy modification
  misc_feature 1..32: note = synthetic sequence

SEQ ID NO: 34 - RNA, 32 nt, synthetic construct; identical to SEQ ID NO: 12
  source 1..32: mol_type = other RNA
  modified_base 1: mod_base = OTHER; note = Methoxy modification
  modified_base 1..2: mod_base = OTHER; note = Thiophosphate ester subunit connection
  modified_base 2: mod_base = OTHER; note = Methoxy modification
  modified_base 2..3: mod_base = OTHER; note = Thiophosphate ester subunit connection
  modified_base 3: mod_base = OTHER; note = Methoxy modification
  modified_base 4: mod_base = OTHER; note = Methoxy modification
  modified_base 5: mod_base = OTHER; note = Methoxy modification
  modified_base 6: mod_base = OTHER; note = Methoxy modification
  modified_base 7: mod_base = OTHER; note = Methoxy modification
  modified_base 8: mod_base = OTHER; note = Methoxy modification
  modified_base 9: mod_base = OTHER; note = Methoxy modification
  modified_base 10: mod_base = OTHER; note = Methoxy modification
  modified_base 11: mod_base = OTHER; note = Methoxy modification
  modified_base 12: mod_base = OTHER; note = Methoxy modification
  modified_base 13: mod_base = OTHER; note = Methoxy modification
  modified_base 14: mod_base = OTHER; note = Methoxy modification
  modified_base 15: mod_base = OTHER; note = Methoxy modification
  modified_base 16: mod_base = OTHER; note = Methoxy modification
  modified_base 17: mod_base = OTHER; note = Methoxy modification
  modified_base 18: mod_base = OTHER; note = Methoxy modification
  modified_base 19: mod_base = OTHER; note = Methoxy modification
  modified_base 20: mod_base = OTHER; note = Methoxy modification
  modified_base 21: mod_base = OTHER; note = Methoxy modification
  modified_base 22: mod_base = OTHER; note = Methoxy modification
  modified_base 23: mod_base = OTHER; note = Methoxy modification
  modified_base 24: mod_base = OTHER; note = Methoxy modification
  modified_base 25: mod_base = OTHER; note = Methoxy modification
  modified_base 26: mod_base = OTHER; note = Methoxy modification
  modified_base 27: mod_base = OTHER; note = Methoxy modification
  modified_base 28: mod_base = OTHER; note = Methoxy modification
  modified_base 29: mod_base = OTHER; note = Methoxy modification
  modified_base 30: mod_base = OTHER; note = Methoxy modification
  modified_base 30..31: mod_base = OTHER; note = Thiophosphate ester subunit connection
  modified_base 31: mod_base = OTHER; note = Methoxy modification
  modified_base 31..32: mod_base = OTHER; note = Thiophosphate ester subunit connection
  modified_base 32: mod_base = OTHER; note = Methoxy modification
  misc_feature 1..32: note = synthetic sequence

SEQ ID NO: 35 - RNA, 24 nt, synthetic construct
  source 1..24: mol_type = other RNA
  modified_base 1: mod_base = OTHER; note = Methoxy modification
  modified_base 1..2: mod_base = OTHER; note = Thiophosphate ester subunit connection
  modified_base 2: mod_base = OTHER; note = Methoxy modification
  modified_base 2..3: mod_base = OTHER; note = Thiophosphate ester subunit connection
  modified_base 3: mod_base = OTHER; note = Methoxy modification
  modified_base 4: mod_base = OTHER; note = Methoxy modification
  modified_base 5: mod_base = OTHER; note = Methoxy modification
  modified_base 6: mod_base = OTHER; note = Methoxy modification
  modified_base 7: mod_base = OTHER; note = Methoxy modification
  modified_base 8: mod_base = OTHER; note = Methoxy modification
  modified_base 9: mod_base = OTHER; note = Methoxy modification
  modified_base 10: mod_base = OTHER; note = Methoxy modification
  modified_base 11: mod_base = OTHER; note = Methoxy modification
  modified_base 12: mod_base = OTHER; note = Methoxy modification
  modified_base 13: mod_base = OTHER; note = Methoxy modification
  modified_base 14: mod_base = OTHER; note = Methoxy modification
  modified_base 15: mod_base = OTHER; note = Methoxy modification
  modified_base 16: mod_base = OTHER; note = Methoxy modification
  modified_base 17: mod_base = OTHER; note = Methoxy modification
  modified_base 18: mod_base = OTHER; note = Methoxy modification
  modified_base 19: mod_base = OTHER; note = Methoxy modification
  modified_base 20: mod_base = OTHER; note = Methoxy modification
  modified_base 21: mod_base = OTHER; note = Methoxy modification
  modified_base 22: mod_base = OTHER; note = Methoxy modification
  modified_base 22..23: mod_base = OTHER; note = Thiophosphate ester subunit connection
  modified_base 23: mod_base = OTHER; note = Methoxy modification
  modified_base 23..24: mod_base = OTHER; note = Thiophosphate ester subunit connection
  modified_base 24: mod_base = OTHER; note = Methoxy modification
  misc_feature 1..24: note = synthetic sequence
ctggagttcagacgtgttgctctt

SEQ ID NO: 36 - RNA, 32 nt, synthetic construct; identical to SEQ ID NO: 13
  source 1..32: mol_type = other RNA
  modified_base 1: mod_base = OTHER; note = Methoxy modification
  modified_base 1..2: mod_base = OTHER; note = Thiophosphate ester subunit connection
  modified_base 2: mod_base = OTHER; note = Methoxy modification
  modified_base 2..3: mod_base = OTHER; note = Thiophosphate ester subunit connection
  modified_base 3: mod_base = OTHER; note = Methoxy modification
  modified_base 4: mod_base = OTHER; note = Methoxy modification
  modified_base 5: mod_base = OTHER; note = Methoxy modification
  modified_base 6: mod_base = OTHER; note = Methoxy modification
  modified_base 7: mod_base = OTHER; note = Methoxy modification
  modified_base 8: mod_base = OTHER; note = Methoxy modification
  modified_base 9: mod_base = OTHER; note = Methoxy modification
  modified_base 10: mod_base = OTHER; note = Methoxy modification
  modified_base 11: mod_base = OTHER; note = Methoxy modification
  modified_base 12: mod_base = OTHER; note = Methoxy modification
  modified_base 13: mod_base = OTHER; note = Methoxy modification
  modified_base 14: mod_base = OTHER; note = Methoxy modification
  modified_base 15: mod_base = OTHER; note = Methoxy modification
  modified_base 16: mod_base = OTHER; note = Methoxy modification
  modified_base 17: mod_base = OTHER; note = Methoxy modification
  modified_base 18: mod_base = OTHER; note = Methoxy modification
  modified_base 19: mod_base = OTHER; note = Methoxy modification
  modified_base 20: mod_base = OTHER; note = Methoxy modification
  modified_base 21: mod_base = OTHER; note = Methoxy modification
  modified_base 22: mod_base = OTHER; note = Methoxy modification
  modified_base 23: mod_base = OTHER; note = Methoxy modification
  modified_base 24: mod_base = OTHER; note = Methoxy modification
  modified_base 25: mod_base = OTHER; note = Methoxy modification
  modified_base 26: mod_base = OTHER; note = Methoxy modification
  modified_base 27: mod_base = OTHER; note = Methoxy modification
  modified_base 28: mod_base = OTHER; note = Methoxy modification
  modified_base 29: mod_base = OTHER; note = Methoxy modification
  modified_base 30: mod_base = OTHER; note = Methoxy modification
  modified_base 30..31: mod_base = OTHER; note = Thiophosphate ester subunit connection
  modified_base 31: mod_base = OTHER; note = Methoxy modification
  modified_base 31..32: mod_base = OTHER; note = Thiophosphate ester subunit connection
  modified_base 32: mod_base = OTHER; note = Methoxy modification
  misc_feature 1..32: note = synthetic sequence

SEQ ID NO: 37 - RNA, 24 nt, synthetic construct
  source 1..24: mol_type = other RNA
  modified_base 1: mod_base = OTHER; note = Methoxy modification
  modified_base 1..2: mod_base = OTHER; note = Thiophosphate ester subunit connection
  modified_base 2: mod_base = OTHER; note = Methoxy modification
  modified_base 2..3: mod_base = OTHER; note = Thiophosphate ester subunit connection
  modified_base 3: mod_base = OTHER; note = Methoxy modification
  modified_base 4: mod_base = OTHER; note = Methoxy modification
  modified_base 5: mod_base = OTHER; note = Methoxy modification
  modified_base 6: mod_base = OTHER; note = Methoxy modification
  modified_base 7: mod_base = OTHER; note = Methoxy modification
  modified_base 8: mod_base = OTHER; note = Methoxy modification
  modified_base 9: mod_base = OTHER; note = Methoxy modification
  modified_base 10: mod_base = OTHER; note = Methoxy modification
  modified_base 11: mod_base = OTHER; note = Methoxy modification
  modified_base 12: mod_base = OTHER; note = Methoxy modification
  modified_base 13: mod_base = OTHER; note = Methoxy modification
  modified_base 14: mod_base = OTHER; note = Methoxy modification
  modified_base 15: mod_base = OTHER; note = Methoxy modification
  modified_base 16: mod_base = OTHER; note = Methoxy modification
  modified_base 17: mod_base = OTHER; note = Methoxy modification
  modified_base 18: mod_base = OTHER; note = Methoxy modification
  modified_base 19: mod_base = OTHER; note = Methoxy modification
  modified_base 20: mod_base = OTHER; note = Methoxy modification
  modified_base 21: mod_base = OTHER; note = Methoxy modification
  modified_base 22: mod_base = OTHER; note = Methoxy modification
  modified_base 22..23: mod_base = OTHER; note = Thiophosphate ester subunit connection
  modified_base 23: mod_base = OTHER; note = Methoxy modification
  modified_base 23..24: mod_base = OTHER; note = Thiophosphate ester subunit connection
  modified_base 24: mod_base = OTHER; note = Methoxy modification
  misc_feature 1..24: note = synthetic sequence
ctggagttcagacgttgtgctctt

SEQ ID NO: 38 - RNA, 32 nt, synthetic construct; identical to SEQ ID NO: 14
  source 1..32: mol_type = other RNA
  modified_base 1: mod_base = OTHER; note = Methoxy modification
  modified_base 1..2: mod_base = OTHER; note = Thiophosphate ester subunit connection
  modified_base 2: mod_base = OTHER; note = Methoxy modification
  modified_base 2..3: mod_base = OTHER; note = Thiophosphate ester subunit connection
  modified_base 3: mod_base = OTHER; note = Methoxy modification
  modified_base 4: mod_base = OTHER; note = Methoxy modification
  modified_base 5: mod_base = OTHER; note = Methoxy modification
  modified_base 6: mod_base = OTHER; note = Methoxy modification
  modified_base 7: mod_base = OTHER; note = Methoxy modification
  modified_base 8: mod_base = OTHER; note = Methoxy modification
  modified_base 9: mod_base = OTHER; note = Methoxy modification
  modified_base 10: mod_base = OTHER; note = Methoxy modification
  modified_base 11: mod_base = OTHER; note = Methoxy modification
  modified_base 12: mod_base = OTHER; note = Methoxy modification
  modified_base 13: mod_base = OTHER; note = Methoxy modification
  modified_base 14: mod_base = OTHER; note = Methoxy modification
  modified_base 15: mod_base = OTHER; note = Methoxy modification
  modified_base 16: mod_base = OTHER; note = Methoxy modification
  modified_base 17: mod_base = OTHER; note = Methoxy modification
  modified_base 18: mod_base = OTHER; note = Methoxy modification
  modified_base 19: mod_base = OTHER; note = Methoxy modification
  modified_base 20: mod_base = OTHER; note = Methoxy modification
  modified_base 21: mod_base = OTHER; note = Methoxy modification
  modified_base 22: mod_base = OTHER; note = Methoxy modification
  modified_base 23: mod_base = OTHER; note = Methoxy modification
  modified_base 24: mod_base = OTHER; note = Methoxy modification
  modified_base 25: mod_base = OTHER; note = Methoxy modification
  modified_base 26: mod_base = OTHER; note = Methoxy modification
  modified_base 27: mod_base = OTHER; note = Methoxy modification
  modified_base 28: mod_base = OTHER; note = Methoxy modification
  modified_base 29: mod_base = OTHER; note = Methoxy modification
  modified_base 30: mod_base = OTHER; note = Methoxy modification
  modified_base 30..31: mod_base = OTHER; note = Thiophosphate ester subunit connection
  modified_base 31: mod_base = OTHER; note = Methoxy modification
  modified_base 31..32: mod_base = OTHER; note = Thiophosphate ester subunit connection
  modified_base 32: mod_base = OTHER; note = Methoxy modification
  misc_feature 1..32: note = synthetic sequence

SEQ ID NO: 39 - RNA, 24 nt, synthetic construct
  source 1..24: mol_type = other RNA
  modified_base 1: mod_base = OTHER; note = Methoxy modification
  modified_base 1..2: mod_base = OTHER; note = Thiophosphate ester subunit connection
  modified_base 2: mod_base = OTHER; note = Methoxy modification
  modified_base 2..3: mod_base = OTHER; note = Thiophosphate ester subunit connection
  modified_base 3: mod_base = OTHER; note = Methoxy modification
  modified_base 4: mod_base = OTHER; note = Methoxy modification
  modified_base 5: mod_base = OTHER; note = Methoxy modification
  modified_base 6: mod_base = OTHER; note = Methoxy modification
  modified_base 7: mod_base = OTHER; note = Methoxy modification
  modified_base 8: mod_base = OTHER; note = Methoxy modification
  modified_base 9: mod_base = OTHER; note = Methoxy modification
  modified_base 10: mod_base = OTHER; note = Methoxy modification
  modified_base 11: mod_base = OTHER; note = Methoxy modification
  modified_base 12: mod_base = OTHER; note = Methoxy modification
  modified_base 13: mod_base = OTHER; note = Methoxy modification
  modified_base 14: mod_base = OTHER; note = Methoxy modification
  modified_base 15: mod_base = OTHER; note = Methoxy modification
  modified_base 16: mod_base = OTHER; note = Methoxy modification
  modified_base 17: mod_base = OTHER; note = Methoxy modification
  modified_base 18: mod_base = OTHER; note = Methoxy modification
  modified_base 19: mod_base = OTHER; note = Methoxy modification
  modified_base 20: mod_base = OTHER; note = Methoxy modification
  modified_base 21: mod_base = OTHER; note = Methoxy modification
  modified_base 22: mod_base = OTHER; note = Methoxy modification
  modified_base 22..23: mod_base = OTHER; note = Thiophosphate ester subunit connection
  modified_base 23: mod_base = OTHER; note = Methoxy modification
  modified_base 23..24: mod_base = OTHER; note = Thiophosphate ester subunit connection
  modified_base 24: mod_base = OTHER; note = Methoxy modification
  misc_feature 1..24: note = synthetic sequence
ctggagttcagaccgtgtgctctt

SEQ ID NO: 40 - RNA, 17 nt, synthetic construct
  source 1..17: mol_type = other RNA
  misc_feature 1..17: note = synthetic sequence
gtacattctagatagcc

SEQ ID NO: 41 - RNA, 17 nt, synthetic construct
  source 1..17: mol_type = other RNA
  misc_feature 1..17: note = synthetic sequence
ggctatctagaatgtac

SEQ ID NO: 42 - RNA, 17 nt, synthetic construct
  source 1..17: mol_type = other RNA
  modified_base 1: mod_base = OTHER; note = Methoxy modification
  modified_base 2: mod_base = OTHER; note = Fluorinated modification
  modified_base 3: mod_base = OTHER; note = Methoxy modification
  modified_base 4: mod_base = OTHER; note = Fluorinated modification
  modified_base 5: mod_base = OTHER; note = Methoxy modification
  modified_base 6: mod_base = OTHER; note = Fluorinated modification
  modified_base 7: mod_base = OTHER; note = Fluorinated modification
  modified_base 8: mod_base = OTHER; note = Fluorinated modification
  modified_base 9: mod_base = OTHER; note = Fluorinated modification
  modified_base 10: mod_base = OTHER; note = Methoxy modification
  modified_base 11: mod_base = OTHER; note = Methoxy modification
  modified_base 12: mod_base = OTHER; note = Methoxy modification
  modified_base 13: mod_base = OTHER; note = Fluorinated modification
  modified_base 14: mod_base = OTHER; note = Methoxy modification
  modified_base 15: mod_base = OTHER; note = Methoxy modification
  modified_base 16: mod_base = OTHER; note = Fluorinated modification
  modified_base 17: mod_base = OTHER; note = Fluorinated modification
  misc_feature 1..17: note = synthetic sequence
gtacattctagatagcc

SEQ ID NO: 43 - RNA, 17 nt, synthetic construct
  source 1..17: mol_type = other RNA
  modified_base 1: mod_base = OTHER; note = Methoxy modification
  modified_base 2: mod_base = OTHER; note = Methoxy modification
  modified_base 3: mod_base = OTHER; note = Fluorinated modification
  modified_base 4: mod_base = OTHER; note = Fluorinated modification
  modified_base 5: mod_base = OTHER; note = Methoxy modification
  modified_base 6: mod_base = OTHER; note = Fluorinated modification
  modified_base 7: mod_base = OTHER; note = Fluorinated modification
  modified_base 8: mod_base = OTHER; note = Fluorinated modification
  modified_base 9: mod_base = OTHER; note = Methoxy modification
  modified_base 10: mod_base = OTHER; note = Methoxy modification
  modified_base 11: mod_base = OTHER; note = Methoxy modification
  modified_base 12: mod_base = OTHER; note = Methoxy modification
  modified_base 13: mod_base = OTHER; note = Fluorinated modification
  modified_base 14: mod_base = OTHER; note = Methoxy modification
  modified_base 15: mod_base = OTHER; note = Fluorinated modification
  modified_base 16: mod_base = OTHER; note = Methoxy modification
  modified_base 17: mod_base = OTHER; note = Fluorinated modification
  misc_feature 1..17: note = synthetic sequence
ggctatctagaatgtac

SEQ ID NO: 44 - RNA, 24 nt, synthetic construct
  source 1..24: mol_type = other RNA
  modified_base 1: mod_base = OTHER; note = Methoxy modification
  modified_base 2: mod_base = OTHER; note = Methoxy modification
  modified_base 3: mod_base = OTHER; note = Methoxy modification
  modified_base 4: mod_base = OTHER; note = Methoxy modification
  modified_base 5: mod_base = OTHER; note = Methoxy modification
  modified_base 6: mod_base = OTHER; note = Methoxy modification
  modified_base 7: mod_base = OTHER; note = Methoxy modification
  modified_base 8: mod_base = OTHER; note = Methoxy modification
  modified_base 9: mod_base = OTHER; note = Methoxy modification
  modified_base 10: mod_base = OTHER; note = Methoxy modification
  modified_base 11: mod_base = OTHER; note = Methoxy modification
  modified_base 12: mod_base = OTHER; note = Methoxy modification
  modified_base 13: mod_base = OTHER; note = Methoxy modification
  modified_base 14: mod_base = OTHER; note = Methoxy modification
  modified_base 15: mod_base = OTHER; note = Methoxy modification
  modified_base 16: mod_base = OTHER; note = Methoxy modification
  modified_base 17: mod_base = OTHER; note = Methoxy modification
  modified_base 18: mod_base = OTHER; note = Methoxy modification
  modified_base 19: mod_base = OTHER; note = Methoxy modification
  modified_base 20: mod_base = OTHER; note = Methoxy modification
  modified_base 21: mod_base = OTHER; note = Methoxy modification
  modified_base 22: mod_base = OTHER; note = Methoxy modification
  modified_base 23: mod_base = OTHER; note = Methoxy modification
  modified_base 24: mod_base = OTHER; note = Methoxy modification
  misc_feature 1..24: note = synthetic sequence
ggacatggattcttgtctgtgtcc